European Patent Application EP 4 282 966 A1, published November 29, 2023. Title: OLIGONUCLEOTIDES CONJUGATED TO OLEIC ACID AND USES THEREOF. Applicant: ARTHEX BIOTECH S.L. The sequence listing filed with the application follows.

SEQUENCE LISTING (111 sequences)

SEQ ID NO: 1 - DNA, 15 bp, synthetic construct
  misc_feature 1..15: note = Antagonist of the human hsa-miR-218-5p
  source 1..15: mol_type = other DNA
ttagatcaagcacaa

SEQ ID NO: 2 - DNA, 16 bp, synthetic construct
  misc_feature 1..16: note = Antagonist of the human hsa-miR-23b-3p
  source 1..16: mol_type = other DNA
atccctggcaatgtga

SEQ ID NO: 3 - DNA, 16 bp, synthetic construct
  misc_feature 1..16: note = MD23b-2 V2 3'OI
  misc_feature 1: note = /note="LNA modified base"
  misc_feature 1: note = /note="nucleotide bond by a Phosphorothioate linkage"
  misc_feature 2: note = /note="LNA modified base"
  misc_feature 2: note = /note="nucleotide bond by a Phosphorothioate linkage"
  misc_feature 3: note = /note="nucleotide bond by a Phosphorothioate linkage"
  misc_feature 3: note = /note="5-Methyl-2'-O-Methyl cytidine "
  misc_feature 4: note = /note="nucleotide bond by a Phosphorothioate linkage"
  misc_feature 4: note = /note="5-Methyl-2'-O-Methyl cytidine "
  misc_feature 5: note = /note="2'-O-MOE RNA nucleotide"
  misc_feature 6: note = /note="LNA modified base"
  misc_feature 7: note = /note="nucleotide bond by a Phosphorothioate linkage"
  misc_feature 7: note = /note="2'-O-MOE RNA nucleotide"
  misc_feature 8: note = /note="nucleotide bond by a Phosphorothioate linkage"
  misc_feature 8: note = /note="2 -O-Methyl-nucleotide"
  misc_feature 9: note = /note="LNA modified base"
  misc_feature 9: note = /note="nucleotide bond by a Phosphorothioate linkage"
  misc_feature 9: note = /note="2'-O-MOE RNA nucleotide"
  misc_feature 11: note = /note="LNA modified base"
  misc_feature 11: note = /note="2'-O-MOE RNA nucleotide"
  misc_feature 12: note = /note="LNA modified base"
  misc_feature 14: note = /note="LNA modified base"
  misc_feature 14: note = /note="nucleotide bond by a Phosphorothioate linkage"
  misc_feature 14: note = /note="2'-O-MOE RNA nucleotide"
  misc_feature 15: note = /note="LNA modified base"
  misc_feature 15: note = /note="nucleotide bond by a Phosphorothioate linkage"
  misc_feature 16: note = /note="nucleotide conjugated to NHC6 conjugated to oleic acid"
  source 1..16: mol_type = other DNA
atccctggcaatgtga

SEQ ID NO: 4 - DNA, 16 bp, synthetic construct
  misc_feature 1..16: note = MD23b-2-PS/PO 3'OI
  misc_feature 1: note = /note="nucleotide bond by a Phosphorothioate linkage"
  misc_feature 1: note = /note="LNA nucleotide"
  misc_feature 2: note = /note="2'-O-MOE RNA nucleotides "
  misc_feature 3: note = /note="5-Methyl-2'-O-Methyl cytidine"
  misc_feature 4: note = /note="5-Methyl-2'-O-Methyl cytidine"
  misc_feature 5: note = /note="5-Methyl-2'-O-Methyl cytidine"
  misc_feature 6: note = /note="nucleotide bond by a Phosphorothioate linkage"
  misc_feature 6: note = /note="LNA nucleotide"
  misc_feature 7: note = /note="2 -O-Methyl-nucleotide"
  misc_feature 8: note = /note="2 -O-Methyl-nucleotide"
  misc_feature 9: note = /note="nucleotide bond by a Phosphorothioate linkage"
  misc_feature 9: note = /note="5-Methyl-2'-O-Methyl cytidine"
  misc_feature 10: note = /note="LNA nucleotide"
  misc_feature 11: note = /note="nucleotide bond by a Phosphorothioate linkage"
  misc_feature 11: note = /note="2'-O-MOE RNA nucleotides "
  misc_feature 12: note = /note="nucleotide bond by a Phosphorothioate linkage"
  misc_feature 12: note = /note="LNA nucleotide"
  misc_feature 13: note = /note="LNA nucleotide"
  misc_feature 14: note = /note="nucleotide bond by a Phosphorothioate linkage"
  misc_feature 14: note = /note="2'-O-MOE RNA nucleotides "
  misc_feature 15: note = /note="nucleotide bond by a Phosphorothioate linkage"
  misc_feature 15: note = /note="LNA nucleotide"
  misc_feature 16: note = /note="LNA nucleotide"
  misc_feature 16: note = /note="nucleotide conjugated to NHC6 conjugated to oleic acid"
  source 1..16: mol_type = other DNA
atccctggcaatgtga

SEQ ID NO: 5 - DNA, 16 bp, synthetic construct
  misc_feature 1..16: note = MD23b-2-PS/PO 5'OI
  misc_feature 1: note = /note="nucleotide conjugated to NHC6 conjugated to oleic acid"
  misc_feature 1: note = /note="nucleotide bond by a Phosphorothioate linkage"
  misc_feature 1: note = /note="LNA nucleotide"
  misc_feature 2: note = /note="2'-O-MOE RNA nucleotides "
  misc_feature 3: note = /note="5-Methyl-2'-O-Methyl cytidine"
  misc_feature 4: note = /note="5-Methyl-2'-O-Methyl cytidine"
  misc_feature 5: note = /note="5-Methyl-2'-O-Methyl cytidine"
  misc_feature 6: note = /note="nucleotide bond by a Phosphorothioate linkage"
  misc_feature 6: note = /note="LNA nucleotide"
  misc_feature 7: note = /note="2 -O-Methyl-nucleotide"
  misc_feature 8: note = /note="2 -O-Methyl-nucleotide"
  misc_feature 9: note = /note="nucleotide bond by a Phosphorothioate linkage"
  misc_feature 9: note = /note="5-Methyl-2'-O-Methyl cytidine"
  misc_feature 10: note = /note="LNA nucleotide"
  misc_feature 11: note = /note="nucleotide bond by a Phosphorothioate linkage"
  misc_feature 11: note = /note="2'-O-MOE RNA nucleotides "
  misc_feature 12: note = /note="nucleotide bond by a Phosphorothioate linkage"
  misc_feature 12: note = /note="LNA nucleotide"
  misc_feature 13: note = /note="LNA nucleotide"
  misc_feature 14: note = /note="nucleotide bond by a Phosphorothioate linkage"
  misc_feature 14: note = /note="2'-O-MOE RNA nucleotides "
  misc_feature 15: note = /note="nucleotide bond by a Phosphorothioate linkage"
  misc_feature 15: note = /note="LNA nucleotide"
  misc_feature 16: note = /note="LNA nucleotide"
  source 1..16: mol_type = other DNA
atccctggcaatgtga

SEQ ID NO: 6 - DNA, 16 bp, synthetic construct
  misc_feature 1..16: note = MD23b-2-PS/PO
  misc_feature 1: note = /note="nucleotide bond by a Phosphorothioate linkage"
  misc_feature 1: note = /note="LNA nucleotide"
  misc_feature 2: note = /note="2'-O-MOE RNA nucleotides "
  misc_feature 3: note = /note="5-Methyl-2'-O-Methyl cytidine"
  misc_feature 4: note = /note="5-Methyl-2'-O-Methyl cytidine"
  misc_feature 5: note = /note="5-Methyl-2'-O-Methyl cytidine"
  misc_feature 6: note = /note="nucleotide bond by a Phosphorothioate linkage"
  misc_feature 6: note = /note="LNA nucleotide"
  misc_feature 7: note = /note="2 -O-Methyl-nucleotide"
  misc_feature 8: note = /note="2 -O-Methyl-nucleotide"
  misc_feature 9: note = /note="nucleotide bond by a Phosphorothioate linkage"
  misc_feature 9: note = /note="5-Methyl-2'-O-Methyl cytidine"
  misc_feature 10: note = /note="LNA nucleotide"
  misc_feature 11: note = /note="nucleotide bond by a Phosphorothioate linkage"
  misc_feature 11: note = /note="2'-O-MOE RNA nucleotides "
  misc_feature 12: note = /note="nucleotide bond by a Phosphorothioate linkage"
  misc_feature 12: note = /note="LNA nucleotide"
  misc_feature 13: note = /note="LNA nucleotide"
  misc_feature 14: note = /note="nucleotide bond by a Phosphorothioate linkage"
  misc_feature 14: note = /note="2'-O-MOE RNA nucleotides "
  misc_feature 15: note = /note="nucleotide bond by a Phosphorothioate linkage"
  misc_feature 15: note = /note="LNA nucleotide"
  misc_feature 16: note = /note="LNA nucleotide"
  source 1..16: mol_type = other DNA
atccctggcaatgtga

SEQ ID NO: 7 - DNA, 15 bp, synthetic construct
  misc_feature 1..15: note = 218 MOE Oleic 3'
  misc_feature 1: note = /note="nucleotide bond by a Phosphorothioate linkage"
  misc_feature 1: note = /note="LNA modified base"
  misc_feature 2: note = /note="nucleotide bond by a Phosphorothioate linkage"
  misc_feature 2: note = /note="LNA modified base"
  misc_feature 3: note = /note="nucleotide bond by a Phosphorothioate linkage"
  misc_feature 3: note = /note="2'-O-MOE RNA nucleotides"
  misc_feature 4: note = /note="nucleotide bond by a Phosphorothioate linkage"
  misc_feature 4: note = /note="LNA modified base"
  misc_feature 5: note = /note="nucleotide bond by a Phosphorothioate linkage"
  misc_feature 5: note = /note="2'-O-MOE RNA nucleotides"
  misc_feature 6: note = /note="nucleotide bond by a Phosphorothioate linkage"
  misc_feature 6: note = /note="2'-O-MOE RNA nucleotides"
  misc_feature 7: note = /note="LNA modified base"
  misc_feature 8: note = /note="nucleotide bond by a Phosphorothioate linkage"
  misc_feature 8: note = /note="2'-O-MOE RNA nucleotides"
  misc_feature 9: note = /note="2'-O-MOE RNA nucleotides"
  misc_feature 10: note = /note="LNA modified base"
  misc_feature 11: note = /note="2'-O-MOE RNA nucleotides"
  misc_feature 12: note = /note="nucleotide bond by a Phosphorothioate linkage"
  misc_feature 12: note = /note="LNA modified base"
  misc_feature 13: note = /note="nucleotide bond by a Phosphorothioate linkage"
  misc_feature 13: note = /note="2'-O-MOE RNA nucleotides"
  misc_feature 14: note = /note="nucleotide bond by a Phosphorothioate linkage"
  misc_feature 14: note = /note="LNA modified base"
  misc_feature 15: note = /note="LNA modified base"
  misc_feature 15: note = /note="nucleotide conjugated to NHC6 conjugated to oleic acid"
  source 1..15: mol_type = other DNA
ttagatcaagcacaa

SEQ ID NO: 8 - DNA, 15 bp, synthetic construct
  misc_feature 1..15: note = 218 MOE DD Oleic 3'
  misc_feature 1: note = /note="LNA modified base"
  misc_feature 1: note = /note="nucleotide bond by a Phosphorothioate linkage"
  misc_feature 2: note = /note="LNA modified base"
  misc_feature 2: note = /note="nucleotide bond by a Phosphorothioate linkage"
  misc_feature 3: note = /note="nucleotide bond by a Phosphorothioate linkage"
  misc_feature 3: note = /note="2'-O-MOE RNA nucleotides"
  misc_feature 4: note = /note="LNA modified base"
  misc_feature 4: note = /note="nucleotide bond by a Phosphorothioate linkage"
  misc_feature 5: note = /note="nucleotide bond by a Phosphorothioate linkage"
  misc_feature 5: note = /note="2'-O-MOE RNA nucleotides"
  misc_feature 6: note = /note="nucleotide bond by a Phosphorothioate linkage"
  misc_feature 6: note = /note="2'-O-MOE RNA nucleotides"
  misc_feature 7: note = /note="LNA modified base"
  misc_feature 8: note = /note="nucleotide bond by a Phosphorothioate linkage"
  misc_feature 8: note = /note="2'-O-MOE RNA nucleotides"
  misc_feature 9: note = /note="nucleotide bond by a Phosphorothioate linkage"
  misc_feature 9: note = /note="2'-O-MOE RNA nucleotides"
  misc_feature 10: note = /note="LNA modified base"
  misc_feature 11: note = /note="2'-O-MOE RNA nucleotides"
  misc_feature 12: note = /note="LNA modified base"
  misc_feature 12: note = /note="nucleotide bond by a Phosphorothioate linkage"
  misc_feature 13: note = /note="nucleotide bond by a Phosphorothioate linkage"
  misc_feature 13: note = /note="2'-O-MOE RNA nucleotides"
  misc_feature 14: note = /note="nucleotide bond by a Phosphorothioate linkage"
  misc_feature 14: note = /note="2'-O-Methyl-2,6-diaminopurine "
  misc_feature 15: note = /note="2'-O-Methyl-2,6-diaminopurine "
  misc_feature 15: note = /note="nucleotide conjugated to NHC6 conjugated to oleic acid"
  source 1..15: mol_type = other DNA
ttagatcaagcacaa

SEQ ID NO: 9 - DNA, 15 bp, synthetic construct
  misc_feature 1..15: note = 218 OME/MOE oleic 3'
  misc_feature 1: note = /note="nucleotide bond by a Phosphorothioate linkage"
  misc_feature 1: note = /note="LNA modified base"
  misc_feature 2: note = /note="nucleotide bond by a Phosphorothioate linkage"
  misc_feature 2: note = /note="2'-O-MOE RNA nucleotides"
  misc_feature 3: note = /note="nucleotide bond by a Phosphorothioate linkage"
  misc_feature 3: note = /note="2 -O-Methyl-nucleotides"
  misc_feature 4: note = /note="nucleotide bond by a Phosphorothioate linkage"
  misc_feature 4: note = /note="LNA modified base"
  misc_feature 4: note = /note="2 -O-Methyl-nucleotides"
  misc_feature 5: note = /note="nucleotide bond by a Phosphorothioate linkage"
  misc_feature 6: note = /note="nucleotide bond by a Phosphorothioate linkage"
  misc_feature 6: note = /note="2 -OMe-5-methyluridine or 2 -OMe-ribothymidine "
  misc_feature 7: note = /note="LNA modified base"
  misc_feature 8: note = /note="nucleotide bond by a Phosphorothioate linkage"
  misc_feature 8: note = /note="2'-O-MOE RNA nucleotides"
  misc_feature 9: note = /note="2'-O-MOE RNA nucleotides"
  misc_feature 10: note = /note="LNA modified base"
  misc_feature 11: note = /note="2'-O-MOE RNA nucleotides"
  misc_feature 12: note = /note="nucleotide bond by a Phosphorothioate linkage"
  misc_feature 12: note = /note="LNA modified base"
  misc_feature 13: note = /note="nucleotide bond by a Phosphorothioate linkage"
  misc_feature 13: note = /note="2'-O-MOE RNA nucleotides"
  misc_feature 14: note = /note="nucleotide bond by a Phosphorothioate linkage"
  misc_feature 14: note = /note="2'-O-MOE RNA nucleotides"
  misc_feature 15: note = /note="LNA modified base"
  misc_feature 15: note = /note="nucleotide conjugated to NHC6 conjugated to oleic acid"
  source 1..15: mol_type = other DNA
ttagatcaagcacaa

SEQ ID NO: 10 - RNA, 21 nt, synthetic construct
  misc_feature 1..21: note = hsa-miR-218-5p
  source 1..21: mol_type = other RNA
ttgtgcttgatctaaccatgt

SEQ ID NO: 11 - RNA, 23 nt, synthetic construct
  misc_feature 1..23: note = hsa-miR-23b-3p
  source 1..23: mol_type = other RNA
atcacattgccagggattaccac

SEQ ID NO: 12-13 - skipped (2 entries)

SEQ ID NO: 14 - DNA, 15 bp, synthetic construct
  misc_feature 1..15: note = 218 OME/MOE oleic 3'2
  misc_feature 1: note = /note="nucleotide bond by a Phosphorothioate linkage"
  misc_feature 1: note = /note="LNA modified base"
  misc_feature 2: note = /note="nucleotide bond by a Phosphorothioate linkage"
  misc_feature 2: note = /note="LNA modified base"
  misc_feature 3: note = /note="nucleotide bond by a Phosphorothioate linkage"
  misc_feature 3: note = /note="2 -O-Methyl-nucleotides"
  misc_feature 4: note = /note="nucleotide bond by a Phosphorothioate linkage"
  misc_feature 4: note = /note="LNA modified base"
  misc_feature 5: note = /note="nucleotide bond by a Phosphorothioate linkage"
  misc_feature 5: note = /note="2 -O-Methyl-nucleotides"
  misc_feature 6: note = /note="nucleotide bond by a Phosphorothioate linkage"
  misc_feature 6: note = /note="2 -OMe-5-methyluridine or 2 -OMe-ribothymidine"
  misc_feature 7: note = /note="LNA modified base"
  misc_feature 8: note = /note="nucleotide bond by a Phosphorothioate linkage"
  misc_feature 8: note = /note="2'-O-MOE RNA nucleotides"
  misc_feature 9: note = /note="2'-O-MOE RNA nucleotides"
  misc_feature 10: note = /note="LNA modified base"
  misc_feature 11: note = /note="2'-O-MOE RNA nucleotides"
  misc_feature 12: note = /note="nucleotide bond by a Phosphorothioate linkage"
  misc_feature 12: note = /note="LNA modified base"
  misc_feature 13: note = /note="nucleotide bond by a Phosphorothioate linkage"
  misc_feature 13: note = /note="2'-O-MOE RNA nucleotides"
  misc_feature 14: note = /note="nucleotide bond by a Phosphorothioate linkage"
  misc_feature 14: note = /note="2'-O-MOE RNA nucleotides"
  misc_feature 15: note = /note="LNA modified base"
  misc_feature 15: note = /note="nucleotide conjugated to NHC6 conjugated to oleic acid"
  source 1..15: mol_type = other DNA
ttagatcaagcacaa

SEQ ID NO: 15 - DNA, 15 bp, synthetic construct
  misc_feature 1..15: note = 218 MOE
  misc_feature 1: note = /note="nucleotide bond by a Phosphorothioate linkage"
  misc_feature 1: note = /note="nucleotide bond by a Phosphorothioate linkage"
  misc_feature 1: note = /note="LNA modified base"
  misc_feature 1: note = /note="LNA modified base"
  misc_feature 2: note = /note="nucleotide bond by a Phosphorothioate linkage"
  misc_feature 2: note = /note="nucleotide bond by a Phosphorothioate linkage"
  misc_feature 2: note = /note="LNA modified base"
  misc_feature 2: note = /note="LNA modified base"
  misc_feature 3: note = /note="nucleotide bond by a Phosphorothioate linkage"
  misc_feature 3: note = /note="nucleotide bond by a Phosphorothioate linkage"
  misc_feature 3: note = /note="2'-O-MOE RNA nucleotides"
  misc_feature 3: note = /note="2'-O-MOE RNA nucleotides"
  misc_feature 4: note = /note="nucleotide bond by a Phosphorothioate linkage"
  misc_feature 4: note = /note="nucleotide bond by a Phosphorothioate linkage"
  misc_feature 4: note = /note="LNA modified base"
  misc_feature 4: note = /note="LNA modified base"
  misc_feature 5: note = /note="nucleotide bond by a Phosphorothioate linkage"
  misc_feature 5: note = /note="nucleotide bond by a Phosphorothioate linkage"
  misc_feature 5: note = /note="2'-O-MOE RNA nucleotides"
  misc_feature 5: note = /note="2'-O-MOE RNA nucleotides"
  misc_feature 6: note = /note="nucleotide bond by a Phosphorothioate linkage"
  misc_feature 6: note = /note="nucleotide bond by a Phosphorothioate linkage"
  misc_feature 6: note = /note="2'-O-MOE RNA nucleotides"
  misc_feature 6: note = /note="2'-O-MOE RNA nucleotides"
  misc_feature 7: note = /note="LNA modified base"
  misc_feature 7: note = /note="LNA modified base"
  misc_feature 8: note = /note="nucleotide bond by a Phosphorothioate linkage"
  misc_feature 8: note = /note="nucleotide bond by a Phosphorothioate linkage"
  misc_feature 8: note = /note="2'-O-MOE RNA nucleotides"
  misc_feature 8: note = /note="2'-O-MOE RNA nucleotides"
  misc_feature 9: note = /note="2'-O-MOE RNA nucleotides"
  misc_feature 9: note = /note="2'-O-MOE RNA nucleotides"
  misc_feature 10: note = /note="LNA modified base"
  misc_feature 10: note = /note="LNA modified base"
  misc_feature 11: note = /note="2'-O-MOE RNA nucleotides"
  misc_feature 11: note = /note="2'-O-MOE RNA nucleotides"
  misc_feature 12: note = /note="nucleotide bond by a Phosphorothioate linkage"
  misc_feature 12: note = /note="nucleotide bond by a Phosphorothioate linkage"
  misc_feature 12: note = /note="LNA modified base"
  misc_feature 12: note = /note="LNA modified base"
  misc_feature 13: note = /note="nucleotide bond by a Phosphorothioate linkage"
  misc_feature 13: note = /note="nucleotide bond by a Phosphorothioate linkage"
  misc_feature 13: note = /note="2'-O-MOE RNA nucleotides"
  misc_feature 13: note = /note="2'-O-MOE RNA nucleotides"
  misc_feature 14: note = /note="nucleotide bond by a Phosphorothioate linkage"
  misc_feature 14: note = /note="nucleotide bond by a Phosphorothioate linkage"
  misc_feature 14: note = /note="LNA modified base"
  misc_feature 14: note = /note="LNA modified base"
  misc_feature 15: note = /note="LNA modified base"
  misc_feature 15: note = /note="LNA modified base"
  misc_feature 15: note = /note="nucleotide conjugated to NHC6 conjugated to oleic acid"
  source 1..15: mol_type = other DNA
ttagatcaagcacaa

SEQ ID NO: 16 - DNA, 16 bp, synthetic construct
  misc_feature 1..16: note = MD23b-2 V2 3 Pal
  misc_feature 1: note = /note="LNA modified base"
  misc_feature 1: note = /note="nucleotide bond by a Phosphorothioate linkage"
  misc_feature 2: note = /note="LNA modified base"
  misc_feature 2: note = /note="nucleotide bond by a Phosphorothioate linkage"
  misc_feature 3: note = /note="nucleotide bond by a Phosphorothioate linkage"
  misc_feature 3: note = /note="5-Methyl-2'-O-Methyl cytidine "
  misc_feature 3: note = /note="2 -O-Methyl-nucleotide"
  misc_feature 4: note = /note="nucleotide bond by a Phosphorothioate linkage"
  misc_feature 4: note = /note="5-Methyl-2'-O-Methyl cytidine "
  misc_feature 4: note = /note="2 -O-Methyl-nucleotide"
  misc_feature 5: note = /note="2'-O-MOE RNA nucleotide"
  misc_feature 6: note = /note="LNA modified base"
  misc_feature 7: note = /note="nucleotide bond by a Phosphorothioate linkage"
  misc_feature 7: note = /note="2'-O-MOE RNA nucleotide"
  misc_feature 8: note = /note="nucleotide bond by a Phosphorothioate linkage"
  misc_feature 8: note = /note="2 -O-Methyl-nucleotide"
  misc_feature 9: note = /note="LNA modified base"
  misc_feature 9: note = /note="nucleotide bond by a Phosphorothioate linkage"
  misc_feature 9: note = /note="2'-O-MOE RNA nucleotide"
  misc_feature 11: note = /note="LNA modified base"
  misc_feature 11: note = /note="2'-O-MOE RNA nucleotide"
  misc_feature 12: note = /note="LNA modified base"
  misc_feature 14: note = /note="LNA modified base"
  misc_feature 14: note = /note="nucleotide bond by a Phosphorothioate linkage"
  misc_feature 14: note = /note="2'-O-MOE RNA nucleotide"
  misc_feature 15: note = /note="LNA modified base"
  misc_feature 15: note = /note="nucleotide bond by a Phosphorothioate linkage"
  misc_feature 16: note = /note="nucleotide conjugated to NHC6 conjugated to palmitic acid"
  source 1..16: mol_type = other DNA
atccctggcaatgtga

SEQ ID NO: 17 - DNA, 16 bp, synthetic construct
  misc_feature 1..16: note = MD23b-2 V2
  misc_feature 1: note = /note="LNA modified base"
  misc_feature 1: note = /note="nucleotide bond by a Phosphorothioate linkage"
  misc_feature 2: note = /note="LNA modified base"
  misc_feature 2: note = /note="nucleotide bond by a Phosphorothioate linkage"
  misc_feature 3: note = /note="nucleotide bond by a Phosphorothioate linkage"
  misc_feature 3: note = /note="5-Methyl-2'-O-Methyl cytidine "
  misc_feature 3: note = /note="2 -O-Methyl-nucleotide"
  misc_feature 4: note = /note="nucleotide bond by a Phosphorothioate linkage"
  misc_feature 4: note = /note="5-Methyl-2'-O-Methyl cytidine "
  misc_feature 4: note = /note="2 -O-Methyl-nucleotide"
  misc_feature 5: note = /note="2'-O-MOE RNA nucleotide"
  misc_feature 6: note = /note="LNA modified base"
  misc_feature 7: note = /note="nucleotide bond by a Phosphorothioate linkage"
  misc_feature 7: note = /note="2'-O-MOE RNA nucleotide"
  misc_feature 8: note = /note="nucleotide bond by a Phosphorothioate linkage"
  misc_feature 8: note = /note="2 -O-Methyl-nucleotide"
  misc_feature 9: note = /note="LNA modified base"
  misc_feature 9: note = /note="nucleotide bond by a Phosphorothioate linkage"
  misc_feature 9: note = /note="2'-O-MOE RNA nucleotide"
  misc_feature 11: note = /note="LNA modified base"
  misc_feature 11: note = /note="2'-O-MOE RNA nucleotide"
  misc_feature 12: note = /note="LNA modified base"
  misc_feature 14: note = /note="LNA modified base"
  misc_feature 14: note = /note="nucleotide bond by a Phosphorothioate linkage"
  misc_feature 14: note = /note="2'-O-MOE RNA nucleotide"
  misc_feature 15: note = /note="LNA modified base"
  misc_feature 15: note = /note="nucleotide bond by a Phosphorothioate linkage"
  source 1..16: mol_type = other DNA
atccctggcaatgtga

SEQ ID NO: 18 - DNA, 16 bp, synthetic construct
  misc_feature 1..16: note = MD23 MOE
  misc_feature 1: note = /note="nucleotide bond by a Phosphorothioate linkage"
  misc_feature 1: note = /note="LNA modified base"
  misc_feature 2: note = /note="nucleotide bond by a Phosphorothioate linkage"
  misc_feature 2: note = /note="LNA modified base"
  misc_feature 3: note = /note="nucleotide bond by a Phosphorothioate linkage"
  misc_feature 3: note = /note="2'-O-MOE RNA nucleotides"
  misc_feature 4: note = /note="2'-O-MOE RNA nucleotides"
  misc_feature 5: note = /note="nucleotide bond by a Phosphorothioate linkage"
  misc_feature 5: note = /note="2'-O-MOE RNA nucleotides"
  misc_feature 6: note = /note="nucleotide bond by a Phosphorothioate linkage"
  misc_feature 6: note = /note="2'-O-MOE RNA nucleotides"
  misc_feature 7: note = /note="2'-O-MOE RNA nucleotides"
  misc_feature 8: note = /note="nucleotide bond by a Phosphorothioate linkage"
  misc_feature 8: note = /note="2'-O-MOE RNA nucleotides"
  misc_feature 9: note = /note="2'-O-MOE RNA nucleotides"
  misc_feature 10: note = /note="2'-O-MOE RNA nucleotides"
  misc_feature 11: note = /note="nucleotide bond by a Phosphorothioate linkage"
  misc_feature 11: note = /note="2'-O-MOE RNA nucleotides"
  misc_feature 12: note = /note="LNA modified base"
  misc_feature 13: note = /note="nucleotide bond by a Phosphorothioate linkage"
  misc_feature 13: note = /note="2'-O-MOE RNA nucleotides"
  misc_feature 14: note = /note="2'-O-MOE RNA nucleotides"
  misc_feature 15: note = /note="nucleotide bond by a Phosphorothioate linkage"
  misc_feature 15: note = /note="LNA modified base"
  misc_feature 16: note = /note="LNA modified base"
  source 1..16: mol_type = other DNA
atccctggcaatgtga

SEQ ID NO: 19 - RNA, 97 nt, synthetic construct
  misc_feature 1..97: note = The microRNA precursor (pre-microRNA) of hsa-miR-23b-3p
  source 1..97: mol_type = other RNA
ctcaggtgctctggctgcttgggttcctggcatgctgatttgtgacttaagattaaaatcacattgccagggattaccacgcaaccacgaccttggc

SEQ ID NO: 20 - RNA, 110 nt, synthetic construct
  misc_feature 1..110: note = Pre-hsa-miR-218-5p-1(chr4:20529898-20530007)
  source 1..110: mol_type = other RNA
gtgataatgtagcgagattttctgttgtgcttgatctaaccatgtggttgcgaggtatgagtaaaacatggttccgtcaagcaccatggaacgtcacgcagctttctaca

SEQ ID NO: 21 - RNA, 110 nt, synthetic construct
  misc_feature 1..110: note = Pre-miR-218-2 (chr5:1681951 SI- 168195260)
  source 1..110: mol_type = other RNA
gaccagtcgctgcggggctttcctttgtgcttgatctaaccatgtggtggaacgatggaaacggaacatggttctgtcaagcaccgcggaaagcaccgtgctctcctgca

SEQ ID NO: 22 - DNA, 16 bp, synthetic construct
  misc_feature 1..16: note = MD23b-2 V2 3 OI without specific spacer molecule
  misc_feature 1: note = /note="LNA modified base"
  misc_feature 1: note = /note="nucleotide bond by a Phosphorothioate linkage"
  misc_feature 2: note = /note="LNA modified base"
  misc_feature 2: note = /note="nucleotide bond by a Phosphorothioate linkage"
  misc_feature 3: note = /note="nucleotide bond by a Phosphorothioate linkage"
  misc_feature 3: note = /note="5-Methyl-2'-O-Methyl cytidine "
  misc_feature 3: note = /note="2 -O-Methyl-nucleotide"
  misc_feature 4: note = /note="nucleotide bond by a Phosphorothioate linkage"
  misc_feature 4: note = /note="5-Methyl-2'-O-Methyl cytidine "
  misc_feature 4: note = /note="2 -O-Methyl-nucleotide"
  misc_feature 5: note = /note="2'-O-MOE RNA nucleotide"
  misc_feature 6: note = /note="LNA modified base"
  misc_feature 7: note = /note="nucleotide bond by a Phosphorothioate linkage"
  misc_feature 7: note = /note="2'-O-MOE RNA nucleotide"
  misc_feature 8: note = /note="nucleotide bond by a Phosphorothioate linkage"
  misc_feature 8: note = /note="2 -O-Methyl-nucleotide"
  misc_feature 9: note = /note="LNA modified base"
  misc_feature 9: note = /note="nucleotide bond by a Phosphorothioate linkage"
  misc_feature 9: note = /note="2'-O-MOE RNA nucleotide"
  misc_feature 11: note = /note="LNA modified base"
  misc_feature 11: note = /note="2'-O-MOE RNA nucleotide"
  misc_feature 12: note = /note="LNA modified base"
  misc_feature 14: note = /note="LNA modified base"
  misc_feature 14: note = /note="nucleotide bond by a Phosphorothioate linkage"
  misc_feature 14: note = /note="2'-O-MOE RNA nucleotide"
  misc_feature 15: note = /note="LNA modified base"
  misc_feature 15: note = /note="nucleotide bond by a Phosphorothioate linkage"
  misc_feature 16: note = /note="nucleotide conjugated to a spacer molecule conjugated to oleic acid"
  source 1..16: mol_type = other DNA
atccctggcaatgtga

SEQ ID NO: 23 - DNA, 16 bp, synthetic construct
  misc_feature 1..16: note = MD23b-2-PS/PO 3 OI without specific spacer molecule
  misc_feature 1: note = /note="nucleotide bond by a Phosphorothioate linkage"
  misc_feature 1: note = /note="LNA nucleotide"
  misc_feature 2: note = /note="2'-O-MOE RNA nucleotides "
  misc_feature 3: note = /note="5-Methyl-2'-O-Methyl cytidine"
  misc_feature 4: note = /note="5-Methyl-2'-O-Methyl cytidine"
  misc_feature 5: note = /note="5-Methyl-2'-O-Methyl cytidine"
  misc_feature 6: note = /note="nucleotide bond by a Phosphorothioate linkage"
  misc_feature 6: note = /note="LNA nucleotide"
  misc_feature 7: note = /note="2 -O-Methyl-nucleotide"
  misc_feature 8: note = /note="2 -O-Methyl-nucleotide"
  misc_feature 9: note = /note="nucleotide bond by a Phosphorothioate linkage"
  misc_feature 9: note = /note="5-Methyl-2'-O-Methyl cytidine"
  misc_feature 10: note = /note="LNA nucleotide"
  misc_feature 11: note = /note="nucleotide bond by a Phosphorothioate linkage"
  misc_feature 11: note = /note="2'-O-MOE RNA nucleotides "
  misc_feature 12: note = /note="nucleotide bond by a Phosphorothioate linkage"
  misc_feature 12: note = /note="LNA nucleotide"
  misc_feature 13: note = /note="LNA nucleotide"
  misc_feature 14: note = /note="nucleotide bond by a Phosphorothioate linkage"
  misc_feature 14: note = /note="2'-O-MOE RNA nucleotides "
  misc_feature 15: note = /note="nucleotide bond by a Phosphorothioate linkage"
  misc_feature 15: note = /note="LNA nucleotide"
  misc_feature 16: note = /note="LNA nucleotide"
  misc_feature 16: note = /note="nucleotide conjugated to a Spacer molecule conjugated to oleic acid"
  source 1..16: mol_type = other DNA
atccctggcaatgtga

SEQ ID NO: 24 - DNA, 16 bp, synthetic construct
  misc_feature 1..16: note = MD23b-2-PS/PO 5 OI without specific spacer molecule
  misc_feature 1: note = /note="nucleotide conjugated to a Spacer molecule conjugated to oleic acid"
  misc_feature 1: note = /note="nucleotide bond by a Phosphorothioate linkage"
  misc_feature 1: note = /note="LNA nucleotide"
  misc_feature 2: note = /note="2'-O-MOE RNA nucleotides "
  misc_feature 3: note = /note="5-Methyl-2'-O-Methyl cytidine"
  misc_feature 4: note = /note="5-Methyl-2'-O-Methyl cytidine"
  misc_feature 5: note = /note="5-Methyl-2'-O-Methyl cytidine"
  misc_feature 6: note = /note="nucleotide bond by a Phosphorothioate linkage"
  misc_feature 6: note = /note="LNA nucleotide"
  misc_feature 7: note = /note="2 -O-Methyl-nucleotide"
  misc_feature 8: note = /note="2 -O-Methyl-nucleotide"
  misc_feature 9: note = /note="nucleotide bond by a Phosphorothioate linkage"
  misc_feature 9: note = /note="5-Methyl-2'-O-Methyl cytidine"
  misc_feature 10: note = /note="LNA nucleotide"
  misc_feature 11: note = /note="nucleotide bond by a Phosphorothioate linkage"
  misc_feature 11: note = /note="2'-O-MOE RNA nucleotides "
  misc_feature 12: note = /note="nucleotide bond by a Phosphorothioate linkage"
  misc_feature 12: note = /note="LNA nucleotide"
  misc_feature 13: note = /note="LNA nucleotide"
  misc_feature 14: note = /note="nucleotide bond by a Phosphorothioate linkage"
  misc_feature 14: note = /note="2'-O-MOE RNA nucleotides "
  misc_feature 15: note = /note="nucleotide bond by a Phosphorothioate linkage"
  misc_feature 15: note = /note="LNA nucleotide"
  misc_feature 16: note = /note="LNA nucleotide"
  source 1..16: mol_type = other DNA
atccctggcaatgtga

SEQ ID NO: 25 - DNA, 15 bp, synthetic construct
  misc_feature 1..15: note = 218 MOE Oleic 3 without specific spacer molecule
  misc_feature 1: note = /note="nucleotide bond by a Phosphorothioate linkage"
  misc_feature 1: note = /note="LNA modified base"
  misc_feature 2: note = /note="nucleotide bond by a Phosphorothioate linkage"
  misc_feature 2: note = /note="LNA modified base"
  misc_feature 3: note = /note="nucleotide bond by a Phosphorothioate linkage"
  misc_feature 3: note = /note="2'-O-MOE RNA nucleotides"
  misc_feature 4: note = /note="nucleotide bond by a Phosphorothioate linkage"
  misc_feature 4: note = /note="LNA modified base"
  misc_feature 5: note = /note="nucleotide bond by a Phosphorothioate linkage"
  misc_feature 5: note = /note="2'-O-MOE RNA nucleotides"
  misc_feature 6: note = /note="nucleotide bond by a Phosphorothioate linkage"
  misc_feature 6: note = /note="2'-O-MOE RNA nucleotides"
  misc_feature 7: note = /note="LNA modified base"
  misc_feature 8: note = /note="nucleotide bond by a Phosphorothioate linkage"
  misc_feature 8: note = /note="2'-O-MOE RNA nucleotides"
  misc_feature 9: note = /note="2'-O-MOE RNA nucleotides"
  misc_feature 10: note = /note="LNA modified base"
  misc_feature 11: note = /note="2'-O-MOE RNA nucleotides"
  misc_feature 12: note = /note="nucleotide bond by a Phosphorothioate linkage"
  misc_feature 12: note = /note="LNA modified base"
  misc_feature 13: note = /note="nucleotide bond by a Phosphorothioate linkage"
  misc_feature 13: note = /note="2'-O-MOE RNA nucleotides"
  misc_feature 14: note = /note="nucleotide bond by a Phosphorothioate linkage"
  misc_feature 14: note = /note="LNA modified base"
  misc_feature 15: note = /note="LNA modified base"
  misc_feature 15: note = /note="nucleotide conjugated to a Spacer molecule conjugated to oleic acid"
  source 1..15: mol_type = other DNA
ttagatcaagcacaa

SEQ ID NO: 26 - DNA, 15 bp, synthetic construct
  misc_feature 1..15: note = 218 MOE DD Oleic 3 without specific spacer molecule
  misc_feature 1: note = /note="LNA modified base"
  misc_feature 1: note = /note="nucleotide bond by a Phosphorothioate linkage"
  misc_feature 2: note = /note="LNA modified base"
  misc_feature 2: note = /note="nucleotide bond by a Phosphorothioate linkage"
  misc_feature 3: note = /note="nucleotide bond by a Phosphorothioate linkage"
  misc_feature 3: note = /note="2'-O-MOE RNA nucleotides"
  misc_feature 4: note = /note="LNA modified base"
  misc_feature 4: note = /note="nucleotide bond by a Phosphorothioate linkage"
  misc_feature 5: note = /note="nucleotide bond by a Phosphorothioate linkage"
  misc_feature 5: note = /note="2'-O-MOE RNA nucleotides"
  misc_feature 6: note = /note="nucleotide bond by a Phosphorothioate linkage"
  misc_feature 6: note = /note="2'-O-MOE RNA nucleotides"
  misc_feature 7: note = /note="LNA modified base"
  misc_feature 8: note = /note="nucleotide bond by a Phosphorothioate linkage"
  misc_feature 8: note = /note="2'-O-MOE RNA nucleotides"
  misc_feature 9: note = /note="nucleotide bond by a Phosphorothioate linkage"
  misc_feature 9: note = /note="2'-O-MOE RNA nucleotides"
  misc_feature 10: note = /note="LNA modified base"
  misc_feature 11: note = /note="2'-O-MOE RNA nucleotides"
  misc_feature 12: note = /note="LNA modified base"
  misc_feature 12: note = /note="nucleotide bond by a Phosphorothioate linkage"
  misc_feature 13: note = /note="nucleotide bond by a Phosphorothioate linkage"
  misc_feature 13: note = /note="2'-O-MOE RNA nucleotides"
  misc_feature 14: note = /note="nucleotide bond by a Phosphorothioate linkage"
  misc_feature 14: note = /note="2'-O-Methyl-2,6-diaminopurine "
  misc_feature 15: note = /note="2'-O-Methyl-2,6-diaminopurine "
  misc_feature 15: note = /note="nucleotide conjugated to a Spacer molecule conjugated to oleic acid"
  source 1..15: mol_type = other DNA
ttagatcaagcacaa

SEQ ID NO: 27 - DNA, 15 bp, synthetic construct
  misc_feature 1..15: note = 218 OME/MOE oleic 3 without specific spacer molecule
  misc_feature 1: note = /note="nucleotide bond by a Phosphorothioate linkage"
  misc_feature 1: note = /note="LNA modified base"
  misc_feature 2: note = /note="nucleotide bond by a Phosphorothioate linkage"
  misc_feature 2: note = /note="2'-O-MOE RNA nucleotides"
  misc_feature 3: note = /note="nucleotide bond by a Phosphorothioate linkage"
  misc_feature 3: note = /note="2 -O-Methyl-nucleotides"
  misc_feature 4: note = /note="nucleotide bond by a Phosphorothioate linkage"
  misc_feature 4: note = /note="LNA modified base"
  misc_feature 4: note = /note="2 -O-Methyl-nucleotides"
  misc_feature 5: note = /note="nucleotide bond by a Phosphorothioate linkage"
  misc_feature 6: note = /note="nucleotide bond by a Phosphorothioate linkage"
  misc_feature 6: note = /note="2 -OMe-5-methyluridine or 2 -OMe-ribothymidine "
  misc_feature 7: note = /note="LNA modified base"
  misc_feature 8: note = /note="nucleotide bond by a Phosphorothioate linkage"
  misc_feature 8: note = /note="2'-O-MOE RNA nucleotides"
  misc_feature 9: note = /note="2'-O-MOE RNA nucleotides"
  misc_feature 10: note = /note="LNA modified base"
  misc_feature 11: note = /note="2'-O-MOE RNA nucleotides"
  misc_feature 12: note = /note="nucleotide bond by a Phosphorothioate linkage"
  misc_feature 12: note = /note="LNA modified base"
  misc_feature 13: note = /note="nucleotide bond by a Phosphorothioate linkage"
  misc_feature 13: note = /note="2'-O-MOE RNA nucleotides"
  misc_feature 14: note = /note="nucleotide bond by a Phosphorothioate linkage"
  misc_feature 14: note = /note="2'-O-MOE RNA nucleotides"
  misc_feature 15: note = /note="LNA modified base"
  misc_feature 15: note = /note="nucleotide conjugated to a spacer molecule conjugated to oleic acid"
  source 1..15: mol_type = other DNA
ttagatcaagcacaa

SEQ ID NO: 28 - DNA, 15 bp, synthetic construct
  misc_feature 1..15: note = 218 OME/MOE oleic 3 2 without specific spacer molecule
  misc_feature 1: note = /note="nucleotide bond by a Phosphorothioate linkage"
  misc_feature 1: note = /note="LNA modified base"
  misc_feature 2: note = /note="nucleotide bond by a Phosphorothioate linkage"
  misc_feature 2: note = /note="LNA modified base"
  misc_feature 3: note = /note="nucleotide bond by a Phosphorothioate linkage"
  misc_feature 3: note = /note="2 -O-Methyl-nucleotides"
  misc_feature 4: note = /note="nucleotide bond by a Phosphorothioate linkage"
  misc_feature 4: note = /note="LNA modified base"
  misc_feature 5: note = /note="nucleotide bond by a Phosphorothioate linkage"
  misc_feature 5: note = /note="2 -O-Methyl-nucleotides"
  misc_feature 6: note = /note="nucleotide bond by a Phosphorothioate linkage"
  misc_feature 6: note = /note="2 -OMe-5-methyluridine or 2 -OMe-ribothymidine"
  misc_feature 7: note = /note="LNA modified base"
  misc_feature 8: note = /note="nucleotide bond by a Phosphorothioate linkage"
  misc_feature 8: note = /note="2'-O-MOE RNA nucleotides"
  misc_feature 9: note = /note="2'-O-MOE RNA nucleotides"
  misc_feature 10: note = /note="LNA modified base"
  misc_feature 11: note = /note="2'-O-MOE RNA nucleotides"
  misc_feature 12: note = /note="nucleotide bond by a Phosphorothioate linkage"
  misc_feature 12: note = /note="LNA modified base"
  misc_feature 13: note = /note="nucleotide bond by a Phosphorothioate linkage"
  misc_feature 13: note = /note="2'-O-MOE RNA nucleotides"
  misc_feature 14: note = /note="nucleotide bond by a Phosphorothioate linkage"
  misc_feature 14: note = /note="2'-O-MOE RNA nucleotides"
  misc_feature 15: note = /note="LNA modified base"
  misc_feature 15: note = /note="nucleotide conjugated to a Spacer molecule conjugated to oleic acid"
  source 1..15: mol_type = other DNA
ttagatcaagcacaa

SEQ ID NO: 29 - DNA, 16 bp, synthetic construct
  misc_feature 1..16: note = MD23b-2 V2 3 Pal without specific spacer molecule
  misc_feature 1: note = /note="LNA modified base"
  misc_feature 1: note = /note="nucleotide bond by a Phosphorothioate linkage"
  misc_feature 2: note = /note="LNA modified base"
  misc_feature 2: note = /note="nucleotide bond by a Phosphorothioate linkage"
  misc_feature 3: note = /note="nucleotide bond by a Phosphorothioate linkage"
  misc_feature 3: note = /note="5-Methyl-2'-O-Methyl cytidine "
  misc_feature 3: note = /note="2 -O-Methyl-nucleotide"
  misc_feature 4: note = /note="nucleotide bond by a Phosphorothioate linkage"
  misc_feature 4: note = /note="5-Methyl-2'-O-Methyl cytidine "
  misc_feature 4: note = /note="2 -O-Methyl-nucleotide"
  misc_feature 5: note = /note="2'-O-MOE RNA nucleotide"
  misc_feature 6: note = /note="LNA modified base"
  misc_feature 7: note = /note="nucleotide bond by a Phosphorothioate linkage"
  misc_feature 7: note = /note="2'-O-MOE RNA nucleotide"
  misc_feature 8: note = /note="nucleotide bond by a Phosphorothioate linkage"
  misc_feature 8: note = /note="2 -O-Methyl-nucleotide"
  misc_feature 9: note = /note="LNA modified base"
  misc_feature 9: note = /note="nucleotide bond by a Phosphorothioate linkage"
  misc_feature 9: note = /note="2'-O-MOE RNA nucleotide"
  misc_feature 11: note = /note="LNA modified base"
  misc_feature 11: note = /note="2'-O-MOE RNA nucleotide"
  misc_feature 12: note = /note="LNA modified base"
  misc_feature 14: note = /note="LNA modified base"
  misc_feature 14: note = /note="nucleotide bond by a Phosphorothioate linkage"
  misc_feature 14: note = /note="2'-O-MOE RNA nucleotide"
  misc_feature 15: note = /note="LNA modified base"
  misc_feature 15: note = /note="nucleotide bond by a Phosphorothioate linkage"
  misc_feature 16: note = /note="nucleotide conjugated to a spacer molecule conjugated to palmitic acid"
  source 1..16: mol_type = other DNA
atccctggcaatgtga

SEQ ID NO: 30 - DNA, 20 bp, synthetic construct
  misc_feature 1..20: note = Gapdh Fwd
  source 1..20: mol_type = other DNA
atcaacgggaagcccatcac

SEQ ID NO: 31 - DNA, 21 bp, synthetic construct
  misc_feature 1..21: note = Gapdh Rv
  source 1..21: mol_type = other DNA
cttccacaatgccaaagttgt

SEQ ID NO: 32 - DNA, 23 bp, synthetic construct
  misc_feature 1..23: note = Atp2a Fwd
  source 1..23: mol_type = other DNA
gctcatggtcctcaagatctcac

SEQ ID NO: 33 - DNA, 20 bp, synthetic construct
  misc_feature 1..20: note = Atp2a Rv
  source 1..20: mol_type = other DNA
gggtcagtgcctcagctttg

SEQ ID NO: 34 - DNA, 21 bp, synthetic construct
  misc_feature 1..21: note = Clcn1 Fwd
  source 1..21: mol_type = other DNA
gtcctcagcaagtttatgtcc

SEQ ID NO: 35 - DNA, 20 bp, synthetic construct
  misc_feature 1..20: note = Clcn1 Rv
  source 1..20: mol_type = other DNA
gaatcctcgccagtaattcc

SEQ ID NO: 36 - DNA, 20 bp, synthetic construct
  misc_feature 1..20: note = Nfix Fwd
  source 1..20: mol_type = other DNA
tcgacgacagtgagatggag

SEQ ID NO: 37 - DNA, 20 bp, synthetic construct
  misc_feature 1..20: note = Nfix Rv
  source 1..20: mol_type = other DNA
caaactccttcagcgagtcc

SEQ ID NO: 38 - DNA, 25 bp, synthetic construct
  misc_feature 1..25: note = Mbnl1 ex5 F
  source 1..25: mol_type = other DNA
aggggagatgctctcgggaaaagtg

SEQ ID NO: 39 - DNA, 32 bp, synthetic construct
  misc_feature 1..32: note = Mbnl1 ex5 R
  source 1..32: mol_type = other DNA
gttggctagagcctgttggtattggaaaatac

SEQ ID NO: 40 - DNA, 28 bp, synthetic construct
  misc_feature 1..28: note = Probe Mbnl1: /56
  source 1..28: mol_type = other DNA
tcgcaaatcagctgtgaggagattccct

SEQ ID NO: 41 - DNA, 20 bp, synthetic construct
  misc_feature 1..20: note = Mbnl1 F
  source 1..20: mol_type = other DNA
taccgattgcaccaccaaac

SEQ ID NO: 42 - DNA, 21 bp, synthetic construct
  misc_feature 1..21: note = Mbnl1 R
  source 1..21: mol_type = other DNA
gctgctttcagcaaagttgtc

SEQ ID NO: 43 - DNA, 24 bp, synthetic construct
  misc_feature 1..24: note = Mbnl2 probe
  source 1..24: mol_type = other DNA
cccggcagacagcaccatgatcga

SEQ ID NO: 44 - DNA, 19 bp, synthetic construct
  misc_feature 1..19: note = Mbnl2 F
  source 1..19: mol_type = other DNA
gagacagactgccgctttg

SEQ ID NO: 45 - DNA, 21 bp, synthetic construct
  misc_feature 1..21: note = Mbnl2 R
  source 1..21: mol_type = other DNA
ggttacggtgttgtcgtttgt

SEQ ID NO: 46 - DNA, 21 bp, synthetic construct
  misc_feature 1..21: note = Gapdh probe
  source 1..21: mol_type = other DNA
cgcctggtcaccagggctgct

SEQ ID NO: 47 - DNA, 21 bp, synthetic construct
  misc_feature 1..21: note = Gapdh _For
  source 1..21: mol_type = other DNA
caacggatttggtcgtattgg

SEQ ID NO: 48 - DNA, 25 bp, synthetic construct
  misc_feature 1..25: note = Gapdh _Rev
  source 1..25: mol_type = other DNA
tgatggcaacaatatccactttacc

SEQ ID NO: 49 - DNA, 16 bp, synthetic construct
  misc_feature 1..16: note = MD23b-2 V2 3 OI with C6SSC6 and NHC6
  misc_feature 1: note = /note="LNA modified base"
  misc_feature 1: note = /note="nucleotide bond by a Phosphorothioate linkage"
  misc_feature 2: note = /note="LNA modified base"
  misc_feature 2: note = /note="nucleotide bond by a Phosphorothioate linkage"
  misc_feature 3: note = /note="nucleotide bond by a Phosphorothioate linkage"
  misc_feature 3: note = /note="5-Methyl-2'-O-Methyl cytidine "
  misc_feature 3: note = /note="2 -O-Methyl-nucleotide"
  misc_feature 4: note = /note="nucleotide bond by a Phosphorothioate linkage"
  misc_feature 4: note = /note="5-Methyl-2'-O-Methyl cytidine "
  misc_feature 4: note = /note="2 -O-Methyl-nucleotide"
  misc_feature 5: note = /note="2'-O-MOE RNA nucleotide"
  misc_feature 6: note = /note="LNA modified base"
  misc_feature 7: note = /note="nucleotide bond by a Phosphorothioate linkage"
  misc_feature 7: note = /note="2'-O-MOE RNA nucleotide"
  misc_feature 8: note = /note="nucleotide bond by a Phosphorothioate linkage"
  misc_feature 8: note = /note="2 -O-Methyl-nucleotide"
  misc_feature 9: note = /note="LNA modified base"
  misc_feature 9: note = /note="nucleotide bond by a Phosphorothioate linkage"
  misc_feature 9: note = /note="2'-O-MOE RNA nucleotide"
  misc_feature 11: note = /note="LNA modified base"
  misc_feature 11: note = /note="2'-O-MOE RNA nucleotide"
  misc_feature 12: note = /note="LNA modified base"
  misc_feature 14: note = /note="LNA modified base"
  misc_feature 14: note = /note="nucleotide bond by a Phosphorothioate linkage"
  misc_feature 14: note = /note="2'-O-MOE RNA nucleotide"
  misc_feature 15: note = /note="LNA modified base"
  misc_feature 15: note = /note="nucleotide bond by a Phosphorothioate linkage"
  misc_feature 16: note = /note="nucleotide conjugated to (C6SSC6)(NHC6) conjugated to oleic acid"
  source 1..16: mol_type = other DNA
atccctggcaatgtga

SEQ ID NO: 50 - DNA, 16 bp, synthetic construct
  misc_feature 1..16: note = MD23b-2 V2 3 OI with C6SSC6 and NHC3
  misc_feature 1: note = /note="LNA modified base"
  misc_feature 1: note = /note="nucleotide bond by a Phosphorothioate linkage"
  misc_feature 2: note = /note="LNA modified base"
  misc_feature 2: note = /note="nucleotide bond by a Phosphorothioate linkage"
  misc_feature 3: note = /note="nucleotide bond by a Phosphorothioate linkage"
  misc_feature 3: note = /note="5-Methyl-2'-O-Methyl cytidine "
  misc_feature 3: note = /note="2 -O-Methyl-nucleotide"
  misc_feature 4: note = /note="nucleotide bond by a Phosphorothioate linkage"
  misc_feature 4: note = /note="5-Methyl-2'-O-Methyl cytidine "
  misc_feature 4: note = /note="2 -O-Methyl-nucleotide"
  misc_feature 5: note = /note="2'-O-MOE RNA nucleotide"
  misc_feature 6: note = /note="LNA modified base"
  misc_feature 7: note = /note="nucleotide bond by a Phosphorothioate linkage"
  misc_feature 7: note = /note="2'-O-MOE RNA nucleotide"
  misc_feature 8: note = /note="nucleotide bond by a Phosphorothioate linkage"
  misc_feature 8: note = /note="2 -O-Methyl-nucleotide"
  misc_feature 9: note = /note="LNA modified base"
  misc_feature 9: note = /note="nucleotide bond by a Phosphorothioate linkage"
  misc_feature 9: note = /note="2'-O-MOE RNA nucleotide"
  misc_feature 11: note = /note="LNA modified base"
  misc_feature 11: note = /note="2'-O-MOE RNA nucleotide"
  misc_feature 12: note = /note="LNA modified base"
  misc_feature 14: note = /note="LNA modified base"
  misc_feature 14: note = /note="nucleotide bond by a Phosphorothioate linkage"
  misc_feature 14: note = /note="2'-O-MOE RNA nucleotide"
  misc_feature 15: note = /note="LNA modified base"
  misc_feature 15: note = /note="nucleotide bond by a Phosphorothioate linkage"
  misc_feature 16: note = /note="nucleotide conjugated to (C6SSC6)(NHC3) conjugated to oleic acid"
  source 1..16: mol_type = other DNA
atccctggcaatgtga

SEQ ID NO: 51 - DNA, 16 bp, synthetic construct
  misc_feature 1..16: note = MD23b-2-PS/PO 5 OI without spacer molecule
  misc_feature 1: note = /note="nucleotide conjugated to oleic acid"
  misc_feature 1: note = /note="nucleotide bond by a Phosphorothioate linkage"
  misc_feature 1: note = /note="LNA nucleotide"
  misc_feature 2: note = /note="2'-O-MOE RNA nucleotides "
  misc_feature 3: note = /note="5-Methyl-2'-O-Methyl cytidine"
  misc_feature 4: note = /note="5-Methyl-2'-O-Methyl cytidine"
  misc_feature 5: note = /note="5-Methyl-2'-O-Methyl cytidine"
  misc_feature 6: note = /note="nucleotide bond by a Phosphorothioate linkage"
  misc_feature 6: note = /note="LNA nucleotide"
  misc_feature 7: note = /note="2 -O-Methyl-nucleotide"
  misc_feature 8: note = /note="2 -O-Methyl-nucleotide"
  misc_feature 9: note = /note="nucleotide bond by a Phosphorothioate linkage"
  misc_feature 9: note = /note="5-Methyl-2'-O-Methyl cytidine"
  misc_feature 10: note = /note="LNA nucleotide"
  misc_feature 11: note = /note="nucleotide bond by a Phosphorothioate linkage"
  misc_feature 11: note = /note="2'-O-MOE RNA nucleotides "
  misc_feature 12: note = /note="nucleotide bond by a Phosphorothioate linkage"
  misc_feature 12: note = /note="LNA nucleotide"
  misc_feature 13: note = /note="LNA nucleotide"
  misc_feature 14: note = /note="nucleotide bond by a Phosphorothioate linkage"
  misc_feature 14: note = /note="2'-O-MOE RNA nucleotides "
  misc_feature 15: note = /note="nucleotide bond by a Phosphorothioate linkage"
  misc_feature 15: note = /note="LNA nucleotide"
  misc_feature 16: note = /note="LNA nucleotide"
  source 1..16: mol_type = other DNA
atccctggcaatgtga

SEQ ID NO: 52 - DNA, 16 bp, synthetic construct
  misc_feature 1..16: note = functional equivalent sequence of antimiR-23b-3p
  source 1..16: mol_type = other DNA
ytccctggcaatgtga

SEQ ID NO: 53 - DNA, 16 bp, synthetic construct
  misc_feature 1..16: note = functional equivalent sequence of antimiR-23b-3p
  source 1..16: mol_type = other DNA
atccctygcaatgtga

SEQ ID NO: 54 - DNA, 16 bp, synthetic construct
  misc_feature 1..16: note = functional equivalent sequence of antimiR-23b-3p
  source 1..16: mol_type = other DNA
atccctgycaatgtga

SEQ ID NO: 55 - DNA, 16 bp, synthetic construct
  misc_feature 1..16: note = functional equivalent sequence of antimiR-23b-3p
  source 1..16: mol_type = other DNA
atccctggcyatgtga

SEQ ID NO: 56 - DNA, 16 bp, synthetic construct
  misc_feature 1..16: note = functional equivalent sequence of antimiR-23b-3p
  source 1..16: mol_type = other DNA
atccctggcaytgtga

SEQ ID NO: 57 - DNA, 16 bp, synthetic construct
  misc_feature 1..16: note = functional equivalent sequence of antimiR-23b-3p
  source 1..16: mol_type = other DNA
atccctggcaatytga

SEQ ID NO: 58 - DNA, 16 bp, synthetic construct
  misc_feature 1..16: note = functional equivalent sequence of antimiR-23b-3p
  source 1..16: mol_type = other DNA
atccctggcaatgtya

SEQ ID NO: 59 - DNA, 16 bp, synthetic construct
  misc_feature 1..16: note = functional equivalent sequence of antimiR-23b-3p
  source 1..16: mol_type = other DNA
atccctggcaatgtgy

SEQ ID NO: 60 - DNA, 16 bp, synthetic construct
  misc_feature 1..16: note = functional equivalent sequence of antimiR-23b-3p
  source 1..16: mol_type = other DNA
gtccctggcaatgtga

SEQ ID NO: 61 - DNA, 16 bp, synthetic construct
  misc_feature 1..16: note = functional equivalent sequence of antimiR-23b-3p
  source 1..16: mol_type = other DNA
  variation 3: note = t=u
attcctggcaatgtga

SEQ ID NO: 62 - DNA, 16 bp, synthetic construct
  misc_feature 1..16: note = functional equivalent sequence of antimiR-23b-3p
  source 1..16: mol_type = other DNA
  variation 4: note = t=u
atctctggcaatgtga

SEQ ID NO: 63 - DNA, 16 bp, synthetic construct
  misc_feature 1..16: note = functional equivalent sequence of antimiR-23b-3p
  source 1..16: mol_type = other DNA
  variation 5: note = t=u
atccttggcaatgtga

SEQ ID NO: 64 - DNA, 16 bp, synthetic construct
  misc_feature 1..16: note = functional equivalent sequence of antimiR-23b-3p
  source 1..16: mol_type = other DNA
  variation 9: note = t=u
atccctggtaatgtga

SEQ ID NO: 65 - DNA, 16 bp, synthetic construct
  misc_feature 1..16: note = functional equivalent sequence of antimiR-23b-3p
  source 1..16: mol_type = other DNA
atccctggcgatgtga

SEQ ID NO: 66 - DNA, 16 bp, synthetic construct
  misc_feature 1..16: note = functional equivalent sequence of antimiR-23b-3p
  source 1..16: mol_type = other DNA
atccctggcagtgtga

SEQ ID NO: 67 - DNA, 16 bp, synthetic construct
  misc_feature 1..16: note = functional equivalent sequence of antimiR-23b-3p
  source 1..16: mol_type = other DNA
atccctggcaatgtgg

SEQ ID NO: 68 - DNA, 16 bp, synthetic construct
  misc_feature 1..16: note = functional equivalent sequence of antimiR-23b-3p
  misc_feature 1: note = /note="n = hypoxanthine "
  source 1..16: mol_type = other DNA
ntccctggcaatgtga

SEQ ID NO: 69 - DNA, 16 bp, synthetic construct
  misc_feature 1..16: note = functional equivalent sequence of antimiR-23b-3p
  misc_feature 10: note = /note="n = hypoxanthine "
  source 1..16: mol_type = other DNA
atccctggcnatgtga

SEQ ID NO: 70 - DNA, 16 bp, synthetic construct
  misc_feature 1..16: note = functional equivalent sequence of antimiR-23b-3p
  misc_feature 11: note = /note="n = hypoxanthine "
  source 1..16: mol_type = other DNA
atccctggcantgtga

SEQ ID NO: 71 - DNA, 16 bp, synthetic construct
  misc_feature 1..16: note = functional equivalent sequence of antimiR-23b-3p
  misc_feature 16: note = /note="n = hypoxanthine "
  source 1..16: mol_type = other DNA
atccctggcaatgtgn

SEQ ID NO: 72 - DNA, 16 bp, synthetic construct
  misc_feature 1..16: note = functional equivalent sequence of antimiR-23b-3p
  misc_feature 2: note = /note="n = hypoxanthine "
  source 1..16: mol_type = other DNA
anccctggcaatgtga

SEQ ID NO: 73 - DNA, 16 bp, synthetic construct
  misc_feature 1..16: note = functional equivalent sequence of antimiR-23b-3p
  misc_feature 6: note = /note="n = hypoxanthine "
  source 1..16: mol_type = other DNA
atcccnggcaatgtga

SEQ ID NO: 74 - DNA, 16 bp, synthetic construct
  misc_feature 1..16: note = functional equivalent sequence of antimiR-23b-3p
  misc_feature 12: note = /note="n = hypoxanthine "
  source 1..16: mol_type = other DNA
atccctggcaangtga

SEQ ID NO: 75 - DNA, 16 bp, synthetic construct
  misc_feature 1..16: note = functional equivalent sequence of antimiR-23b-3p
  misc_feature 14: note = /note="n = hypoxanthine "
  source 1..16: mol_type = other DNA
atccctggcaatgnga

SEQ ID NO: 76 - DNA, 16 bp, synthetic construct
  misc_feature 1..16: note = functional equivalent sequence of antimiR-23b-3p
  misc_feature 7: note = /note="n = hypoxanthine "
  source 1..16: mol_type = other DNA
atccctngcaatgtga

SEQ ID NO: 77 - DNA, 16 bp, synthetic construct
  misc_feature 1..16: note = functional equivalent sequence of antimiR-23b-3p
  misc_feature 8: note = /note="n = hypoxanthine "
  source 1..16: mol_type = other DNA
atccctgncaatgtga

SEQ ID NO: 78 - DNA, 16 bp, synthetic construct
  misc_feature 1..16: note = functional equivalent sequence of antimiR-23b-3p
  misc_feature 13: note = /note="n = hypoxanthine "
  source 1..16: mol_type = other DNA
atccctggcaatntga

SEQ ID NO: 79 - DNA, 16 bp, synthetic construct
  misc_feature 1..16: note = functional equivalent sequence of antimiR-23b-3p
  misc_feature 15: note = /note="n = hypoxanthine "
  source 1..16: mol_type = other DNA
atccctggcaatgtna

SEQ ID NO: 80 - DNA, 15 bp, synthetic construct
  misc_feature 1..15: note = functional equivalent sequence of antimiR-218-5p
  source 1..15: mol_type = other DNA
ttygatcaagcacaa

SEQ ID NO: 81 - DNA, 15 bp, synthetic construct
  misc_feature 1..15: note = functional equivalent sequence of antimiR-218-5p
  source 1..15: mol_type = other DNA
ttayatcaagcacaa

SEQ ID NO: 82 - DNA, 15 bp, synthetic construct
  misc_feature 1..15: note = functional equivalent sequence of antimiR-218-5p
  source 1..15: mol_type = other DNA
ttagytcaagcacaa

SEQ ID NO: 83 - DNA, 15 bp, synthetic construct
  misc_feature 1..15: note = functional equivalent sequence of antimiR-218-5p
  source 1..15: mol_type = other DNA
ttagatcyagcacaa

SEQ ID NO: 84 - DNA, 15 bp, synthetic construct
  misc_feature 1..15: note = functional equivalent sequence of antimiR-218-5p
  source 1..15: mol_type = other DNA
ttagatcaygcacaa

SEQ ID NO: 85 - DNA, 15 bp, synthetic construct
  misc_feature 1..15: note = functional equivalent sequence of antimiR-218-5p
  source 1..15: mol_type = other DNA
ttagatcaaycacaa

SEQ ID NO: 86 - DNA, 15 bp, synthetic construct
  misc_feature 1..15: note = functional equivalent sequence of antimiR-218-5p
  source 1..15: mol_type = other DNA
ttagatcaagcycaa

SEQ ID NO: 87 - DNA, 15 bp, synthetic construct
  misc_feature 1..15: note = functional equivalent sequence of antimiR-218-5p
  source 1..15: mol_type = other DNA
ttagatcaagcacya

SEQ ID NO: 88 - DNA, 15 bp, synthetic construct
  misc_feature 1..15: note = functional equivalent sequence of antimiR-218-5p
  source 1..15: mol_type = other DNA
ttagatcaagcacay

SEQ ID NO: 89 - DNA, 15 bp, synthetic construct
  misc_feature 1..15: note = functional equivalent sequence of antimiR-218-5p
  source 1..15: mol_type = other DNA
ttggatcaagcacaa

SEQ ID NO: 90 - DNA, 15 bp, synthetic construct
  misc_feature 1..15: note = functional equivalent sequence of antimiR-218-5p
  source 1..15: mol_type = other DNA
ttaggtcaagcacaa

SEQ ID NO: 91 - DNA, 15 bp, synthetic construct
  misc_feature 1..15: note = /note="combined DNA/RNA molecule" /note="functional equivalent sequence of antimiR-218-5p"
  source 1..15: mol_type = other DNA
  variation 7: note = t=u
ttagattaagcacaa

SEQ ID NO: 92 - DNA, 15 bp, synthetic construct
  misc_feature 1..15: note = functional equivalent sequence of antimiR-218-5p
  source 1..15: mol_type = other DNA
ttagatcgagcacaa

SEQ ID NO: 93 - DNA, 15 bp, synthetic construct
  misc_feature 1..15: note = functional equivalent sequence of antimiR-218-5p
  source 1..15: mol_type = other DNA
ttagatcaggcacaa

SEQ ID NO: 94 - DNA, 15 bp, synthetic construct
  misc_feature 1..15: note = functional equivalent sequence of antimiR-218-5p
  source 1..15: mol_type = other DNA
  variation 11: note = t=u
ttagatcaagtacaa

SEQ ID NO: 95 - DNA, 15 bp, synthetic construct
  misc_feature 1..15: note = functional equivalent sequence of antimiR-218-5p
  source 1..15: mol_type = other DNA
ttagatcaagcgcaa

SEQ ID NO: 96 - DNA, 15 bp, synthetic construct
  misc_feature 1..15: note = /note="combined DNA/RNA molecule" /note="functional equivalent sequence of antimiR-218-5p"
  source 1..15: mol_type = other DNA
  variation 13: note = t=u
ttagatcaagcataa

SEQ ID NO: 97 - DNA, 15 bp, synthetic construct
  misc_feature 1..15: note = functional equivalent sequence of antimiR-218-5p
  source 1..15: mol_type = other DNA
ttagatcaagcacga

SEQ ID NO: 98 - DNA, 15 bp, synthetic construct
  misc_feature 1..15: note = functional equivalent sequence of antimiR-218-5p
  source 1..15: mol_type = other DNA
ttagatcaagcacag

SEQ ID NO: 99 - DNA, 15 bp, synthetic construct
  misc_feature 1..15: note = functional equivalent sequence of antimiR-218-5p
  misc_feature 3: note = /note="n = hypoxanthine "
  source 1..15: mol_type = other DNA
ttngatcaagcacaa

SEQ ID NO: 100 - DNA, 15 bp, synthetic construct
  misc_feature 1..15: note = functional equivalent sequence of antimiR-218-5p
  misc_feature 5: note = /note="n = hypoxanthine "
  source 1..15: mol_type = other DNA
ttagntcaagcacaa

SEQ ID NO: 101 - DNA, 15 bp, synthetic construct
  misc_feature 1..15: note = functional equivalent sequence of antimiR-218-5p
  misc_feature 8: note = /note="n = hypoxanthine "
  source 1..15: mol_type = other DNA
ttagatcnagcacaa

SEQ ID NO: 102 - DNA, 15 bp, synthetic construct
  misc_feature 1..15: note = functional equivalent sequence of antimiR-218-5p
  misc_feature 9: note = /note="n = hypoxanthine "
  source 1..15: mol_type = other DNA
ttagatcangcacaa

SEQ ID NO: 103 - DNA, 15 bp, synthetic construct
  misc_feature 1..15: note = functional equivalent sequence of antimiR-218-5p
  misc_feature 12: note = /note="n = hypoxanthine "
  source 1..15: mol_type = other DNA
ttagatcaagcncaa

SEQ ID NO: 104 - DNA, 15 bp, synthetic construct
  misc_feature 1..15: note = functional equivalent sequence of antimiR-218-5p
  misc_feature 14: note = /note="n = hypoxanthine "
  source 1..15: mol_type = other DNA
ttagatcaagcacna

SEQ ID NO: 105 - DNA, 15 bp, synthetic construct
  misc_feature 1..15: note = functional equivalent sequence of antimiR-218-5p
  misc_feature 15: note = /note="n = hypoxanthine "
  source 1..15: mol_type = other DNA
ttagatcaagcacan

SEQ ID NO: 106 - DNA, 15 bp, synthetic construct
  misc_feature 1..15: note = functional equivalent sequence of antimiR-218-5p
  misc_feature 1: note = /note="n = hypoxanthine "
  source 1..15: mol_type = other DNA
ntagatcaagcacaa

SEQ ID NO: 107 - DNA, 15 bp, synthetic construct
  misc_feature 1..15: note = functional equivalent sequence of antimiR-218-5p
  misc_feature 2: note = /note="n = hypoxanthine "
  source 1..15: mol_type = other DNA
tnagatcaagcacaa

SEQ ID NO: 108 - DNA, 15 bp, synthetic construct
  misc_feature 1..15: note = functional equivalent sequence of antimiR-218-5p
  misc_feature 6: note = /note="n = hypoxanthine "
  source 1..15: mol_type = other DNA
ttagancaagcacaa

SEQ ID NO: 109 - DNA, 15 bp, synthetic construct
  misc_feature 1..15: note = functional equivalent sequence of antimiR-218-5p
  misc_feature 4: note = /note="n = hypoxanthine "
  source 1..15: mol_type = other DNA
ttanatcaagcacaa

SEQ ID NO: 110 - DNA, 15 bp, synthetic construct
  misc_feature 1..15: note = functional equivalent sequence of antimiR-218-5p
  misc_feature 10: note = /note="n = hypoxanthine "
  source 1..15: mol_type = other DNA
ttagatcaancacaa

SEQ ID NO: 111 - DNA, 16 bp, unidentified
  source 1..16: mol_type = unassigned DNA
  variation 1: note = Biotin conjugation
  variation 1..16: note = Phosphorotioated RNA
  variation order(1,4,7,10,13,16): note = LNA modification
  variation 16: note = nucleotide conjugated to digoxigenina NHS-ester
tcacattgccagggat